European Patent Application EP 4 530 295 A2, published April 2, 2025. Title: FCRN ANTAGONISTS AND METHODS OF USE. Applicant: argenx BV. The sequence listing filed with the application follows.

SEQUENCE LISTING (27 sequences)

SEQ ID NO: 1 - protein, 221 aa, synthetic construct
CPPCPAPELLGGPSVFLFPPKPKDTLYITREPEVTCVVVDVSHEDPEVKFNWYVDGVEVHNAKTKPREEQYNSTYRVVSVLTVLHQDWLNGKEYKCKVSNKALPAPIEKTISKAKGQPREPQVYTLPPSRDELTKNQVSLTCLVKGFYPSDIAVEWESNGQPENNYKTTPPVLDSDGSFFLYSKLTVDKSRWQQGNVFSCSVMHEALKFHYTQKSLSLSPG

SEQ ID NO: 2 - protein, 227 aa, synthetic construct
DKTHTCPPCPAPELLGGPSVFLFPPKPKDTLYITREPEVTCVVVDVSHEDPEVKFNWYVDGVEVHNAKTKPREEQYNSTYRVVSVLTVLHQDWLNGKEYKCKVSNKALPAPIEKTISKAKGQPREPQVYTLPPSRDELTKNQVSLTCLVKGFYPSDIAVEWESNGQPENNYKTTPPVLDSDGSFFLYSKLTVDKSRWQQGNVFSCSVMHEALKFHYTQKSLSLSPGK

SEQ ID NO: 3 - protein, 226 aa, synthetic construct
DKTHTCPPCPAPELLGGPSVFLFPPKPKDTLYITREPEVTCVVVDVSHEDPEVKFNWYVDGVEVHNAKTKPREEQYNSTYRVVSVLTVLHQDWLNGKEYKCKVSNKALPAPIEKTISKAKGQPREPQVYTLPPSRDELTKNQVSLTCLVKGFYPSDIAVEWESNGQPENNYKTTPPVLDSDGSFFLYSKLTVDKSRWQQGNVFSCSVMHEALKFHYTQKSLSLSPG

SEQ ID NO: 4 - protein, 221 aa, synthetic construct
CPPCPAPELLAGPSVFLFPPKPKDTLMISRTPEVTCVVVDVSHEDPEVKFNWYVDGVEVHNAKTKPREEQYNSTYRVVSVLTVLHQDWLNGKEYKCKVSNKALPAPIEKTISKAKGQPREPQVYTLPPSRDELTKNQVSLTCLVKGFYPSDIAVEWESNGQPENNYKTTPPVLDSDGSFFLYSKLTVDKSRWQQGNVFSCSVMHEALHNHYTQKSLSLSPG

SEQ ID NO: 5 - protein, 227 aa, synthetic construct
DKTHTCPPCPAPELLAGPSVFLFPPKPKDTLMISRTPEVTCVVVDVSHEDPEVKFNWYVDGVEVHNAKTKPREEQYNSTYRVVSVLTVLHQDWLNGKEYKCKVSNKALPAPIEKTISKAKGQPREPQVYTLPPSRDELTKNQVSLTCLVKGFYPSDIAVEWESNGQPENNYKTTPPVLDSDGSFFLYSKLTVDKSRWQQGNVFSCSVMHEALHNHYTQKSLSLSPGK

SEQ ID NO: 6 - protein, 226 aa, synthetic construct
DKTHTCPPCPAPELLAGPSVFLFPPKPKDTLMISRTPEVTCVVVDVSHEDPEVKFNWYVDGVEVHNAKTKPREEQYNSTYRVVSVLTVLHQDWLNGKEYKCKVSNKALPAPIEKTISKAKGQPREPQVYTLPPSRDELTKNQVSLTCLVKGFYPSDIAVEWESNGQPENNYKTTPPVLDSDGSFFLYSKLTVDKSRWQQGNVFSCSVMHEALHNHYTQKSLSLSPG

SEQ ID NO: 7 - protein, 221 aa, synthetic construct
CPPCPAPELLAGPSVFLFPPKPKDTLYITREPEVTCVVVDVSHEDPEVKFNWYVDGVEVHNAKTKPREEQYNSTYRVVSVLTVLHQDWLNGKEYKCKVSNKALPAPIEKTISKAKGQPREPQVYTLPPSRDELTKNQVSLTCLVKGFYPSDIAVEWESNGQPENNYKTTPPVLDSDGSFFLYSKLTVDKSRWQQGNVFSCSVMHEALKFHYTQKSLSLSPG

SEQ ID NO: 8 - protein, 227 aa, synthetic construct
DKTHTCPPCPAPELLAGPSVFLFPPKPKDTLYITREPEVTCVVVDVSHEDPEVKFNWYVDGVEVHNAKTKPREEQYNSTYRVVSVLTVLHQDWLNGKEYKCKVSNKALPAPIEKTISKAKGQPREPQVYTLPPSRDELTKNQVSLTCLVKGFYPSDIAVEWESNGQPENNYKTTPPVLDSDGSFFLYSKLTVDKSRWQQGNVFSCSVMHEALKFHYTQKSLSLSPGK

SEQ ID NO: 9 - protein, 226 aa, synthetic construct
DKTHTCPPCPAPELLAGPSVFLFPPKPKDTLYITREPEVTCVVVDVSHEDPEVKFNWYVDGVEVHNAKTKPREEQYNSTYRVVSVLTVLHQDWLNGKEYKCKVSNKALPAPIEKTISKAKGQPREPQVYTLPPSRDELTKNQVSLTCLVKGFYPSDIAVEWESNGQPENNYKTTPPVLDSDGSFFLYSKLTVDKSRWQQGNVFSCSVMHEALKFHYTQKSLSLSPG

SEQ ID NO: 10 - protein, 221 aa, synthetic construct
CPPCPAPDLLGDDSVFLFPPKPKDTLMISRTPEVTCVVVDVSDEDGEVKFNWYVDGVEVHNAKTKPREEQYNSTYRVVSVLTVLHQDWLNGKEYKCKVSNKALPRPIEKTISKAKGQPREPQVYTLPPSRDELTKNQVSLTCLVKGFYPSDIAVEWESNGQPENNYKTTPPVLDSDGSFFLYSKLTVDKSRWQQGNVFSCSVMHEALHNHYTQKSLSLSPG

SEQ ID NO: 11 - protein, 227 aa, synthetic construct
DKTHTCPPCPAPDLLGDDSVFLFPPKPKDTLMISRTPEVTCVVVDVSDEDGEVKFNWYVDGVEVHNAKTKPREEQYNSTYRVVSVLTVLHQDWLNGKEYKCKVSNKALPRPIEKTISKAKGQPREPQVYTLPPSRDELTKNQVSLTCLVKGFYPSDIAVEWESNGQPENNYKTTPPVLDSDGSFFLYSKLTVDKSRWQQGNVFSCSVMHEALHNHYTQKSLSLSPGK

SEQ ID NO: 12 - protein, 226 aa, synthetic construct
DKTHTCPPCPAPDLLGDDSVFLFPPKPKDTLMISRTPEVTCVVVDVSDEDGEVKFNWYVDGVEVHNAKTKPREEQYNSTYRVVSVLTVLHQDWLNGKEYKCKVSNKALPRPIEKTISKAKGQPREPQVYTLPPSRDELTKNQVSLTCLVKGFYPSDIAVEWESNGQPENNYKTTPPVLDSDGSFFLYSKLTVDKSRWQQGNVFSCSVMHEALHNHYTQKSLSLSPG

SEQ ID NO: 13 - protein, 221 aa, synthetic construct
CPPCPAPDLLGDDSVFLFPPKPKDTLYITREPEVTCVVVDVSDEDGEVKFNWYVDGVEVHNAKTKPREEQYNSTYRVVSVLTVLHQDWLNGKEYKCKVSNKALPRPIEKTISKAKGQPREPQVYTLPPSRDELTKNQVSLTCLVKGFYPSDIAVEWESNGQPENNYKTTPPVLDSDGSFFLYSKLTVDKSRWQQGNVFSCSVMHEALKFHYTQKSLSLSPG

SEQ ID NO: 14 - protein, 227 aa, synthetic construct
DKTHTCPPCPAPDLLGDDSVFLFPPKPKDTLYITREPEVTCVVVDVSDEDGEVKFNWYVDGVEVHNAKTKPREEQYNSTYRVVSVLTVLHQDWLNGKEYKCKVSNKALPRPIEKTISKAKGQPREPQVYTLPPSRDELTKNQVSLTCLVKGFYPSDIAVEWESNGQPENNYKTTPPVLDSDGSFFLYSKLTVDKSRWQQGNVFSCSVMHEALKFHYTQKSLSLSPGK

SEQ ID NO: 15 - protein, 226 aa, synthetic construct
DKTHTCPPCPAPDLLGDDSVFLFPPKPKDTLYITREPEVTCVVVDVSDEDGEVKFNWYVDGVEVHNAKTKPREEQYNSTYRVVSVLTVLHQDWLNGKEYKCKVSNKALPRPIEKTISKAKGQPREPQVYTLPPSRDELTKNQVSLTCLVKGFYPSDIAVEWESNGQPENNYKTTPPVLDSDGSFFLYSKLTVDKSRWQQGNVFSCSVMHEALKFHYTQKSLSLSPG

SEQ ID NO: 16 - protein, 221 aa, synthetic construct
CPPCPAPELLGGPSVFLFPPKPKDTLMISRTPEVTCVVVDVSHEDPEVKFNWYVDGVEVHNAKTKPREEQYNSTYRVVSVLTVLHQDWLNGKEYKCKVSNKALPAPIEKTISKAKGQPREPQVYTLPPSRDELTKNQVSLTCLVKGFYPSDIAVEWESNGQPENNYKTTPPVLDSDGSFFLYSKLTVDKSRWQQGNVFSCSVMHEALKFHYTQKSLSLSPG

SEQ ID NO: 17 - protein, 227 aa, synthetic construct
DKTHTCPPCPAPELLGGPSVFLFPPKPKDTLMISRTPEVTCVVVDVSHEDPEVKFNWYVDGVEVHNAKTKPREEQYNSTYRVVSVLTVLHQDWLNGKEYKCKVSNKALPAPIEKTISKAKGQPREPQVYTLPPSRDELTKNQVSLTCLVKGFYPSDIAVEWESNGQPENNYKTTPPVLDSDGSFFLYSKLTVDKSRWQQGNVFSCSVMHEALKFHYTQKSLSLSPGK

SEQ ID NO: 18 - protein, 226 aa, synthetic construct
DKTHTCPPCPAPELLGGPSVFLFPPKPKDTLMISRTPEVTCVVVDVSHEDPEVKFNWYVDGVEVHNAKTKPREEQYNSTYRVVSVLTVLHQDWLNGKEYKCKVSNKALPAPIEKTISKAKGQPREPQVYTLPPSRDELTKNQVSLTCLVKGFYPSDIAVEWESNGQPENNYKTTPPVLDSDGSFFLYSKLTVDKSRWQQGNVFSCSVMHEALKFHYTQKSLSLSPG

SEQ ID NO: 19 - protein, 221 aa, synthetic construct
CPPCPAPELLAGPSVFLFPPKPKDTLMISRTPEVTCVVVDVSHEDPEVKFNWYVDGVEVHNAKTKPREEQYNSTYRVVSVLTVLHQDWLNGKEYKCKVSNKALPAPIEKTISKAKGQPREPQVYTLPPSRDELTKNQVSLTCLVKGFYPSDIAVEWESNGQPENNYKTTPPVLDSDGSFFLYSKLTVDKSRWQQGNVFSCSVMHEALKFHYTQKSLSLSPG

SEQ ID NO: 20 - protein, 227 aa, synthetic construct
DKTHTCPPCPAPELLAGPSVFLFPPKPKDTLMISRTPEVTCVVVDVSHEDPEVKFNWYVDGVEVHNAKTKPREEQYNSTYRVVSVLTVLHQDWLNGKEYKCKVSNKALPAPIEKTISKAKGQPREPQVYTLPPSRDELTKNQVSLTCLVKGFYPSDIAVEWESNGQPENNYKTTPPVLDSDGSFFLYSKLTVDKSRWQQGNVFSCSVMHEALKFHYTQKSLSLSPGK

SEQ ID NO: 21 - protein, 226 aa, synthetic construct
DKTHTCPPCPAPELLAGPSVFLFPPKPKDTLMISRTPEVTCVVVDVSHEDPEVKFNWYVDGVEVHNAKTKPREEQYNSTYRVVSVLTVLHQDWLNGKEYKCKVSNKALPAPIEKTISKAKGQPREPQVYTLPPSRDELTKNQVSLTCLVKGFYPSDIAVEWESNGQPENNYKTTPPVLDSDGSFFLYSKLTVDKSRWQQGNVFSCSVMHEALKFHYTQKSLSLSPG

SEQ ID NO: 22 - protein, 221 aa, synthetic construct
CPPCPAPDLLGDDSVFLFPPKPKDTLMISRTPEVTCVVVDVSDEDGEVKFNWYVDGVEVHNAKTKPREEQYNSTYRVVSVLTVLHQDWLNGKEYKCKVSNKALPRPIEKTISKAKGQPREPQVYTLPPSRDELTKNQVSLTCLVKGFYPSDIAVEWESNGQPENNYKTTPPVLDSDGSFFLYSKLTVDKSRWQQGNVFSCSVMHEALKFHYTQKSLSLSPG

SEQ ID NO: 23 - protein, 227 aa, synthetic construct
DKTHTCPPCPAPDLLGDDSVFLFPPKPKDTLMISRTPEVTCVVVDVSDEDGEVKFNWYVDGVEVHNAKTKPREEQYNSTYRVVSVLTVLHQDWLNGKEYKCKVSNKALPRPIEKTISKAKGQPREPQVYTLPPSRDELTKNQVSLTCLVKGFYPSDIAVEWESNGQPENNYKTTPPVLDSDGSFFLYSKLTVDKSRWQQGNVFSCSVMHEALKFHYTQKSLSLSPGK

SEQ ID NO: 24 - protein, 226 aa, synthetic construct
DKTHTCPPCPAPDLLGDDSVFLFPPKPKDTLMISRTPEVTCVVVDVSDEDGEVKFNWYVDGVEVHNAKTKPREEQYNSTYRVVSVLTVLHQDWLNGKEYKCKVSNKALPRPIEKTISKAKGQPREPQVYTLPPSRDELTKNQVSLTCLVKGFYPSDIAVEWESNGQPENNYKTTPPVLDSDGSFFLYSKLTVDKSRWQQGNVFSCSVMHEALKFHYTQKSLSLSPG

SEQ ID NO: 25 - protein, 15 aa, synthetic construct
EPKSCDKTHTCPPCP

SEQ ID NO: 26 - DNA, 20 bp, synthetic construct
  source 1..20: mol_type = other DNA
tggagcacgttgatccacgg

SEQ ID NO: 27 - DNA, 20 bp, synthetic construct
  source 1..20: mol_type = other DNA
ttggcagactccccatacct